European Patent Application EP 4 163 392 A1, published April 12, 2023. Title: Methods and kits for diagnosing muscle atrophy. Applicant: Institut national de recherche pour l'agriculture, l'alimentation et l'environnement Centre Hospitalier Universitaire  de Clermont Ferrand Université Clermont Auvergne. The sequence listing filed with the application follows.

SEQUENCE LISTING (48 sequences)

SEQ ID NO: 1 - DNA, 1191 bp, Homo sapiens
atgacgaccttagtgctggataatggagcttacaacgccaaaatcggttacagccatgaaaatgtgtcggttattcctaattgtcagttccggtcaaaaacagcacgtcttaaaacttttactgccaaccagatagatgaaataaaagacccttctggactcttttacatcctcccttttcaaaagggctacttggtgaattgggatgttcagagacaagtttgggattacctttttggaaaagaaatgtatcaggttgattttttagatactaatattattatcactgaaccatactttaacttcacttcaattcaagaatcaatgaatgaaattctatttgaagaataccagtttcaagcagtattaagagtaaatgctggggctctcagtgcacataggtatttccgagataatccttccgaattatgctgtatcattgttgatagtggatattcctttacacatatagttccttattgtagaagtaaaaagaaaaaagaagcaattattcggataaatgtgggaggaaaactcttaaccaatcatctaaaggagatcatatcttacaggcagctacatgttatggatgaaacacatgtgattaatcaagtgaaagaagatgtatgctatgtgtctcaggatttttatagagacatggatattgcaaagttgaaaggagaagaaaatacagtaatgatagactatgtcttgcctgacttcagtacaattaaaaagggcttttgtaagccaagggaagagatggtgttgagtggaaaatacaaatctggggaacaaattcttcgtttggccaatgagagatttgctgttccggaaatactctttaatccttctgatataggcattcaagaaatgggaattccagaagctattgtctattcaattcaaaatctacctgaagaaatgcagccgcatttttttaagaacattgtcttgacaggaggaaattcccttttcccaggatttagggatcgggtttactcagaagttcgatgtcttactccaacagattatgatgtttctgttgtgctgcctgaaaaccctattacttatgcctgggaaggtggaaaattgatatcagagaatgatgattttgaagatatggtggtaacaagagaagattacgaagaaaatggacatagcgtctgtgaagagaaatttgatatttaa

SEQ ID NO: 2 - DNA, 1014 bp, Homo sapiens
atggaccaaaatgaacacagtcactggggaccacatgcaaagggccaatgtgccagcagatctgagctgagaatcatcctggtgggcaaaacaggaactggcaaaagtgctgcagggaacagcatcctcaggaagcaagcatttgaatcgaagctgggttcccagaccttgactaagacttgcagcaaaagtcagggaagctggggaaatagagagattgtcattattgacacaccagatatgttttcttggaaggaccactgtgaagctctgtacaaagaggtgcagaggtgctacttgctctctgcaccaggaccccatgtgctgctcctggtgactcagctgggccgctatacctcacaggaccagcaggctgcacagagggtgaaggagatctttggagaggatgccatgggacacacaattgtcctctttacccacaaggaagacctcaatggtggctccctgatggattacatgcacgactcagataacaaagccctaagcaagctggtggcagcatgtggtgggcgaatctgtgcctttaataaccgtgctgaagggagcaatcaggatgaccaagtgaaggaactaatggactgtattgaggatctgttgatggagaaaaatggtgatcactataccaatgggttgtacagcctaatacagaggtctaaatgtggacctgtgggatcagatgaaagagtaaaggaattcaaacagagccttataaagtacatggaaactcaaagaagttacacagccttggctgaagcaaactgcctaaaaggagccttaatcaaaacacaactgtgtgttttattttgtattcagttgtttctcagattgataattctgtggctttgcatactgcacagcatgtgcaatttgttttgttgcttactctttagtatgtgcaatttattctgcagtttgctgtttattatacccaaaaagttaatgatatttttgagaacagttattagactagaacgcaagactcctaggttatag

SEQ ID NO: 3 - DNA, 954 bp, Homo sapiens
atgcggctgggcccgaggaccgcggcgttggggctgctgctgctgtgcgccgccgcggccggcgccggcaaggccgaggagctgcactacccgctgggcgagcgccgcagcgactacgaccgcgaggcgctgctgggcgtccaggaagatgtggatgaatatgttaaactcggccacgaagagcagcaaaaaagactgcaggcgatcataaagaaaatcgacttggactcagatggctttctcactgaaagtgaactcagttcatggattcagatgtcttttaagcattatgctatgcaagaagcaaaacaacagtttgttgaatatgataaaaacagtgatgatactgtgacttgggatgaatataacattcagatgtatgatcgtgtgattgactttgatgagaacactgctctggatgatgcagaagaggagtcctttaggaagcttcacttaaaggacaagaagcgatttgaaaaagctaaccaggattcaggtcccggtttgagtcttgaagaatttattgcttttgagcatcctgaagaagttgattatatgacggaatttgtcattcaagaagctttagaagaacatgacaaaaatggtgatggatttgttagtttggaagaatttcttggtgattacaggtgggatccaactgcaaatgaagatccagaatggatacttgttgagaaagacagattcgtgaatgattatgacaaagataacgatggcaggcttgatccccaagagctgttaccttgggtagtacctaataatcagggcattgcacaagaggaggcgcttcatctaattgatgaaatggatttgaatggtgacaaaaagctctctgaagaagagattctggaaaacccggacttgtttctcaccagtgaagccacagattatggcagacagctccatgatgactatttctatcatgatgagctttaa

SEQ ID NO: 4 - DNA, 369 bp, Homo sapiens
atggcgccgcagaaagacaggaagcccaagaggtcaacctggaggtttaatttggaccttactcatccagtagaagatggaatttttgattctggaaattttgagcaatttctacgggagaaggttaaagttaatggcaaaactggaaatctcgggaatgttgttcacattgaacgcttcaagaataaaatcacagttgtttctgagaaacagttctctaaaaggtatttgaaataccttaccaagaaataccttaagaagaacaatcttcgtgattggcttcgagtggttgcatctgacaaggagacctacgaacttcgttacttccagattagtcaagatgaagatgaatcagagtcggaggactag

SEQ ID NO: 5 - DNA, 231 bp, Homo sapiens
atgaacagtgtgggggaggcatgcacggacatgaagcgcgagtacgaccagtgcttcaatcgctggttcgccgagaaatttctcaagggggacagctccggggacccgtgcaccgacctcttcaagcgctaccagcagtgtgttcagaaagcaataaaggagaaagagattcctattgaaggactggagttcatgggccatggcaaagaaaagcctgaaaattcttcttga

SEQ ID NO: 6 - DNA, 882 bp, Homo sapiens
atggcgactttttctggcccggctgggccaatcctgtcgcttaatccgcaggaagatgtcgagtttcaaaaggaggtggcgcaggttcgcaagcgcataacccagcgaaaaaaacaagaacaacttactcctggagtagtctatgtgcgccacctacctaacctacttgacgaaacccagatcttttcatatttctcccagtttggcactgtgacacggttcaggctgtccagaagtaaaaggactggaaatagcaaaggctatgcatttgtggagtttgagtctgaggatgttgccaaaatagttgctgaaacaatgaacaactacctgtttggtgaaagactcttggagtgtcattttatgccacctgaaaaagtacataaagaactctttaaagactggaatattccatttaagcagccatcatatccatcagtgaaacggtataatcggaatcggacactaacacaaaagctacggatggaggagcgatttaaaaagaaagaaagattactcaggaagaaattagctaaaaaaggaattgactatgattttccttctttgattttacagaaaacggaaagtatttcaaaaactaatcgtcagacgtctacaaaaggccaggttttacgtaagaagaagaaaaaagtttcaggtactcttgacactcctgagaagactgtggatagccagggccccacaccagtttgtacaccaacatttttggagaggcgaaaatctcaagtggctgaactgaatgatgatgataaagatgatgaaatagttttcaaacagcccatatcctgtgtaaaagaagaaatacaagagactcaaacacctacacattcacggaaaaaaagacgaagaagcagcaatcagtga

SEQ ID NO: 7 - DNA, 729 bp, Homo sapiens
atgtctggctgtgatgctggggagggagactgttgttcccggagatgcggcgcgcaggacaaggagcatccaagatacctgatcccagaactttgcaaacagttttaccatttaggctgggtcactgggactggaggaggaattagcttgaagcatggcgatgaaatctacattgctccttcaggagtgcaaaaggaacgaattcagcctgaagacatgtttgtttgtgatataaatgaaaaggacataagtggaccttcgccatcgaagaagctaaaaaaaagccagtgtactcctcttttcatgaatgcttacacaatgagaggagcaggtgcagtgattcatacccactctaaagctgctgtgatggccacacttctctttccaggacgggagtttaaaattacacatcaagagatgataaaaggaataaagaaatgtacttccggagggtattatagatatgatgatatgttagtggtacccattattgagaatacacctgaggagaagaccctcaaagatagaatggctcatgcaatgaatgaatacccagactcctgtgcagtactggtcagacgtcatggagtatatgtgtggggggaaacatgggagaaggccaaaaccatgtgtgagtgttatgactatttatttgatattgccgtatcaatgaagaaagtaggacttgatccttcacagctcccagttggagaaaatggaattgtctaa

SEQ ID NO: 8 - DNA, 504 bp, Homo sapiens
atgagtgaatggatgaagaaaggccccttagaatggcaagattacatttacaaagaggtccgagtgacagccagtgagaagaatgagtataaaggatgggttttaactacagacccagtctctgccaatattgtccttgtgaacttccttgaagatggcagcatgtctgtgaccggaattatgggacatgctgtgcagactgttgaaactatgaatgaaggggaccatagagtgagggagaagctgatgcatttgttcacgtctggagactgcaaagcatacagcccagaggatctggaagagagaaagaacagcctaaagaaatggcttgagaagaaccacatccccatcactgaacagggagacgctccaaggactctctgtgtggctggggtcctgactatagacccaccatatggtccagaaaattgcagcagctctaatgagattattctgtcgcgtgttcaggatcttattgaaggacatcttacagcttcccaatga

SEQ ID NO: 9 - DNA, 726 bp, Homo sapiens
atgacagattacggcgaggagcagcgcaacgagctggaggccctggagtccatctaccctgactccttcacagtattatcagaaaatccacccagcttcaccattactgtgacgtctgaggctggagaaaatgatgaaactgtccagactaccctcaagtttacatacagtgaaaaatacccagatgaagctcccctttatgaaatattctcccaggaaaatctagaagataatgatgtctcagacattttaaaattactagcattacaggctgaagaaaatcttggtatggtgatgatttttactctagtgacagctgtgcaagaaaaattaaatgaaatagtagatcagataaaactagaagagagaagaaagaacaaaagaaaagaagcagaagaagctgaaaagcaattattccatggtactccagttacaattgagaatttcttaaattggaaagccaagtttgatgcagaactcttggaaattaaaaagaaaaggatgaaagaagaagaacaagcaggaaaaaataaattaagtgggaaacaactatttgaaacagatcataatcttgacacatctgatatccagttcttggaggatgctggaaacaacgtggaggtagatgagtctttgttccaagaaatggatgacttggagctggaggatgatgaagatgatccagactataatcctgctgacccagagagtgactcagctgactaa

SEQ ID NO: 10 - DNA, 1746 bp, Homo sapiens
atgttggagaactatagcaacctcgtgtcagtggggtatcaagccagcaaaccagatgcactcttcaagttggaacaaggagagccatggacagtagaaaatgaaatccacagccaaatctgtccagaaatcaagaaagttgacaatcatctacagatgcactcacaaaagcaaagatgtctgaagagagtggaacaatgccataaacataatgcatttggaaacatcattcatcagaggaaaagtgattttcctttaaggcaaaatcatgatacatttgacttacatgggaaaatactgaaatcaaatttaagtttagtcaaccagaacaaaaggtatgaaatcaagaattctgtgggggttaatggagatgggaaatccttccttcatgccaagcatgaacaatttcataatgaaatgaacttccccgaaggtggaaattctgtgaatacaaattcacaattcattaagcatcagcgaactcaaaacatagataaaccccatgtatgcactgagtgtgggaaggctttcctcaagaagtctcgcctcatctatcatcagagagttcacactggggagaaacctcatggatgcagtatatgtgggaaagccttctccagaaagtccgggctcactgaacaccagagaaaccacacaggagagaaaccctatgaatgcactgaatgtgacaaagcattccgctggaaatcacagctcaatgcacaccagaaaattcatacaggagagaagtcatatatatgcagtgattgtggaaaaggcttcatcaagaagtctcggctcattaatcatcagagagttcatacaggagagaaaccacatggatgcagcctgtgtgggaaggccttctccaaaaggtccaggctcactgaacaccagagaactcatacaggagagaaaccctatgaatgcactgaatgtgacaaagcattccgctggaaatcacagctcaatgcacatcagaaagctcacacaggagagaagtcatatatatgccgtgattgtggaaaaggcttcattcagaagggaaatctcattgtacatcagcgaattcatactggagaaaaaccctatatatgcaatgaatgtggaaaaggcttcatccaaaagggcaacctccttattcatcgacgtactcacactggagagaaaccctatgtatgcaatgaatgtgggaaaggcttcagccagaagacatgtttaatatcccatcagagatttcacacaggaaagacaccctttgtatgtactgagtgtggaaaatcctgctcacacaagtcaggtctcattaaccaccagagaattcacacaggagagaaaccctatacatgcagtgactgtgggaaagctttcagagataaatcatgtctcaacagacatcggagaactcatacaggggagagaccgtatggatgctctgattgtgggaaagctttctcccacttgtcatgccttgtttatcataagggaatgctgcatgcaagagagaaatgtgtaggttcagtcaaattggaaaatccttgctcagagagtcatagcttatcacatacacgtgatctcatacaggataaagactctgttaacatggtgactctgcagatgccttctgtggcagctcagacctcattaactaacagtgcgttccaagcagagagcaaagtagccattgtgagccagcctgttgccagaagttcagtctcagcagatagtagaatttgcacagaataa

SEQ ID NO: 11 - DNA, 927 bp, Homo sapiens
atggcttccagtaacactgtgttgatgcggttggtagcctccgcatattctattgctcaaaaggcaggaatgatagtcagacgtgttattgctgaaggagacctgggtattgtggagaagacctgtgcaacagacctgcagaccaaagctgaccgattggcacagatgagcatatgttcttcattggcccggaaattccccaaactcacaattataggggaagaggatctgccttctgaggaagtggatcaagagctgattgaagacagtcagtgggaagaaatactgaagcaaccatgcccatcgcagtacagtgctattaaagaagaagatctcgtggtctgggttgatcctctggatggaaccaaggaatataccgaaggtcttcttgacaatgtaacagttcttattggaattgcttatgaaggaaaagccatagcaggagttattaaccagccatattacaactatgaggcaggaccagatgctgtgttggggaggacaatctggggagttttaggtttaggcgcctttgggtttcagctgaaagaagtccctgctgggaaacacattatcacaactactcgatcccatagcaacaagttggttactgactgtgttgctgctatgaaccccgatgctgtgctgcgagtaggaggagcaggaaataagattattcagctgattgaaggcaaagcctctgcttatgtatttgcaagtcctggttgtaagaagtgggatacttgtgctccagaagttattttacatgctgtgggaggcaagttaaccgatatccatgggaatgttcttcagtaccacaaggatgtgaagcatatgaactctgcaggagtcctggccacactgaggaattatgactactatgcaagccgagttccagaatctattaaaaatgcacttgttccttaa

SEQ ID NO: 12 - DNA, 1608 bp, Homo sapiens
atggcgtccctttcccttgcacctgttaacatctttaaggcaggagctgatgaagagagagcagagacagctcgtctgacttcttttattggtgccatcgccattggagacttggtaaagagcaccttgggacccaaaggcatggacaaaattcttctaagcagtggacgagatgcctctcttatggtaaccaatgatggtgccactattctaaaaaacattggtgttgacaatccagcagctaaagttttagttgatatgtcaagggttcaagatgatgaagttggtgatggcactacctctgttaccgttttagcagcagaattattaagggaagcagaatctttaattgcaaaaaagattcatccacagaccatcatagcgggttggagagaagccacgaaggctgcaagagaggcgctgttgagttctgcagttgatcatggttccgatgaagttaaattccgtcaagatttaatgaatattgcgggcacaacattatcctcaaaacttcttactcatcacaaagaccactttacaaagttagctgtagaagcagttctcagactgaaaggctctggcaacctggaggcaattcatattatcaagaagctaggaggaagtttggcagattcctatttagatgaaggcttcctgttggataaaaaaattggagtaaatcaaccaaaacgaattgaaaatgctaaaattcttattgcaaatactggtatggatacagacaaaataaagatatttggttcccgggtaagagttgactctacagcaaaggttgcagaaatagaacatgcggaaaaggaaaaaatgaaggagaaagttgaacgtattcttaagcatggaataaattgctttattaacaggcaattaatttataattatcctgaacagctctttggtgctgctggtgtcatggctattgagcatgcagattttgcaggtgtggaacgcctagctcttgtcacaggtggtgaaattgcctctacctttgatcacccagaactggtgaagcttggaagttgcaaacttatcgaggaagtcatgattggagaagacaaactcattcacttttctggggttgcccttggtgaggcttgtaccattgttttgcgtggtgccactcaacaaattttagatgaagcagaaagatcattgcatgatgctctttgtgttcttgcgcaaactgtaaaggactctagaacagtttatggaggaggctgttctgagatgttgatggctcatgctgtgacacagcttgccaatagaacaccaggcaaagaagctgttgcaatggagtcttatgctaaagcactgagaatgttgccaaccatcatagctgacaatgcaggctatgacagtgcagacctggtggcacagctcagggctgctcacagtgaaggcaataccactgctggattggatatgagggaaggcaccattggagatatggctatcctgggtataacagaaagttttcaagtgaagcgacaggttcttctgagtgcagctgaagcagcagaggtgattctgcgtgtggacaacatcatcaaagcggcacccaggaaacgtgtccctgatcaccacccctgttaa

SEQ ID NO: 13 - DNA, 267 bp, Homo sapiens
atggctgcttcccgcttacccccagcgacgctaacgttaaagcagttcgtaagaaggcaacaagttcttctcctctacagaaggattttgcaaacaattcggcaagttccaaatgattctgatcgcaaatacctggaagattgggcaagagaagaattcagaagaaacaaaagtgccaccgaagaggatacaatccggatgatgattactcaaggcaatatgcagctcaaggagttagaaaaaacacttgctttagcaaaatcttaa

SEQ ID NO: 14 - DNA, 20 bp, Artificial Sequence
  Primer
cgccaaaatcggttacagcc

SEQ ID NO: 15 - DNA, 21 bp, Artificial Sequence
  Primer
tcccaattcaccaagtagccc

SEQ ID NO: 16 - DNA, 22 bp, Artificial Sequence
  Primer
gacctgtgggatcagatgaaag

SEQ ID NO: 17 - DNA, 20 bp, Artificial Sequence
  Primer
cttcagccaaggctgtgtaa

SEQ ID NO: 18 - DNA, 20 bp, Artificial Sequence
  Primer
aacactgctctggatgatgc

SEQ ID NO: 19 - DNA, 21 bp, Artificial Sequence
  Primer
actcaaaccgggacctgaatc

SEQ ID NO: 20 - DNA, 21 bp, Artificial Sequence
  Primer
ggcaaaactggaaatctcggg

SEQ ID NO: 21 - DNA, 19 bp, Artificial Sequence
  Primer
atgcaaccactcgaagcca

SEQ ID NO: 22 - DNA, 19 bp, Artificial Sequence
  Primer
gcttcaatcgctggttcgc

SEQ ID NO: 23 - DNA, 21 bp, Artificial Sequence
  Primer
tctgaacacactgctggtagc

SEQ ID NO: 24 - DNA, 20 bp, Artificial Sequence
  Primer
cgcaggaagatgtcgagttt

SEQ ID NO: 25 - DNA, 22 bp, Artificial Sequence
  Primer
gggtttcgtcaagtaggttagg

SEQ ID NO: 26 - DNA, 19 bp, Artificial Sequence
  Primer
cgccatcgaagaagctaaa

SEQ ID NO: 27 - DNA, 20 bp, Artificial Sequence
  Primer
gcagctttagagtgggtatg

SEQ ID NO: 28 - DNA, 21 bp, Artificial Sequence
  Primer
tgcatttgttcacgtctggag

SEQ ID NO: 29 - DNA, 22 bp, Artificial Sequence
  Primer
agtgatggggatgtggttcttc

SEQ ID NO: 30 - DNA, 20 bp, Artificial Sequence
  Primer
atgctggaaacaacgtggag

SEQ ID NO: 31 - DNA, 22 bp, Artificial Sequence
  Primer
ttcatcatcctccagctccaag

SEQ ID NO: 32 - DNA, 20 bp, Artificial Sequence
  Primer
cctgctcacacaagtcaggt

SEQ ID NO: 33 - DNA, 20 bp, Artificial Sequence
  Primer
acaaggcatgacaagtggga

SEQ ID NO: 34 - DNA, 22 bp, Artificial Sequence
  Primer
cacaactactcgatcccatagc

SEQ ID NO: 35 - DNA, 23 bp, Artificial Sequence
  Primer
cttatttcctgctcctcctactc

SEQ ID NO: 36 - DNA, 20 bp, Artificial Sequence
  Primer
ctggtgtcatggctattgag

SEQ ID NO: 37 - DNA, 21 bp, Artificial Sequence
  Primer
gttctgggtgatcaaaggtag

SEQ ID NO: 38 - DNA, 20 bp, Artificial Sequence
  Primer
acctggaagattgggcaaga

SEQ ID NO: 39 - DNA, 21 bp, Artificial Sequence
  Primer
ccttgagctgcatattgcctt

SEQ ID NO: 40 - DNA, 1008 bp, Homo sapiens
atggggaaggtgaaggtcggagtcaacggatttggtcgtattgggcgcctggtcaccagggctgcttttaactctggtaaagtggatattgttgccatcaatgaccccttcattgacctcaactacatggtttacatgttccaatatgattccacccatggcaaattccatggcaccgtcaaggctgagaacgggaagcttgtcatcaatggaaatcccatcaccatcttccaggagcgagatccctccaaaatcaagtggggcgatgctggcgctgagtacgtcgtggagtccactggcgtcttcaccaccatggagaaggctggggctcatttgcaggggggagccaaaagggtcatcatctctgccccctctgctgatgcccccatgttcgtcatgggtgtgaaccatgagaagtatgacaacagcctcaagatcatcagcaatgcctcctgcaccaccaactgcttagcacccctggccaaggtcatccatgacaactttggtatcgtggaaggactcatgaccacagtccatgccatcactgccacccagaagactgtggatggcccctccgggaaactgtggcgtgatggccgcggggctctccagaacatcatccctgcctctactggcgctgccaaggctgtgggcaaggtcatccctgagctagacgggaagctcactggcatggccttccgtgtccccactgccaacgtgtcagtggtggacctgacctgccgtctagaaaaacctgccaaatatgatgacatcaagaaggtggtgaagcaggcgtcggagggccccctcaaaggcatcctgggctacactgagcaccaggtggtctcctctgacttcaacagcgacacccactcctccacctttgacgctggggctggcattgccctcaacgaccactttgtcaagctcatttcctggtatgacaacgaatttggctacagcaacagggtggtggacctcatggcccacatggcctccaaggagtaa

SEQ ID NO: 41 - DNA, 954 bp, Homo sapiens
atgcccagggaagacagggcgacctggaagtccaactacttccttaagatcatccaactattggatgattatccgaaatgtttcattgtgggagcagacaatgtgggctccaagcagatgcagcagatccgcatgtcccttcgcgggaaggctgtggtgctgatgggcaagaacaccatgatgcgcaaggccatccgagggcacctggaaaacaacccagctctggagaaactgctgcctcatatccgggggaatgtgggctttgtgttcaccaaggaggacctcactgagatcagggacatgttgctggccaataaggtgccagctgctgcccgtgctggtgccattgccccatgtgaagtcactgtgccagcccagaacactggtctcgggcccgagaagacctcctttttccaggctttaggtatcaccactaaaatctccaggggcaccattgaaatcctgagtgatgtgcagctgatcaagactggagacaaagtgggagccagcgaagccacgctgctgaacatgctcaacatctcccccttctcctttgggctggtcatccagcaggtgttcgacaatggcagcatctacaaccctgaagtgcttgatatcacagaggaaactctgcattctcgcttcctggagggtgtccgcaatgttgccagtgtctgtctgcagattggctacccaactgttgcatcagtaccccattctatcatcaacgggtacaaacgagtcctggccttgtctgtggagacggattacaccttcccacttgctgaaaaggtcaaggccttcttggctgatccatctgcctttgtggctgctgcccctgtggctgctgccaccacagctgctcctgctgctgctgcagccccagctaaggttgaagccaaggaagagtcggaggagtcggacgaggatatgggatttggtctctttgactaa

SEQ ID NO: 42 - DNA, 1128 bp, Homo sapiens
atggatgatgatatcgccgcgctcgtcgtcgacaacggctccggcatgtgcaaggccggcttcgcgggcgacgatgccccccgggccgtcttcccctccatcgtggggcgccccaggcaccagggcgtgatggtgggcatgggtcagaaggattcctatgtgggcgacgaggcccagagcaagagaggcatcctcaccctgaagtaccccatcgagcacggcatcgtcaccaactgggacgacatggagaaaatctggcaccacaccttctacaatgagctgcgtgtggctcccgaggagcaccccgtgctgctgaccgaggcccccctgaaccccaaggccaaccgcgagaagatgacccagatcatgtttgagaccttcaacaccccagccatgtacgttgctatccaggctgtgctatccctgtacgcctctggccgtaccactggcatcgtgatggactccggtgacggggtcacccacactgtgcccatctacgaggggtatgccctcccccatgccatcctgcgtctggacctggctggccgggacctgactgactacctcatgaagatcctcaccgagcgcggctacagcttcaccaccacggccgagcgggaaatcgtgcgtgacattaaggagaagctgtgctacgtcgccctggacttcgagcaagagatggccacggctgcttccagctcctccctggagaagagctacgagctgcctgacggccaggtcatcaccattggcaatgagcggttccgctgccctgaggcactcttccagccttccttcctgggcatggagtcctgtggcatccacgaaactaccttcaactccatcatgaagtgtgacgtggacatccgcaaagacctgtacgccaacacagtgctgtctggcggcaccaccatgtaccctggcattgccgacaggatgcagaaggagatcactgccctggcacccagcacaatgaagatcaagatcattgctcctcctgagcgcaagtactccgtgtggatcggcggctccatcctggcctcgctgtccaccttccagcagatgtggatcagcaagcaggagtatgacgagtccggcccctccatcgtccaccgcaaatgcttctag

SEQ ID NO: 43 - DNA, 21 bp, Artificial Sequence
  Primer
aggtcatccctgagctagacg

SEQ ID NO: 44 - DNA, 20 bp, Artificial Sequence
  Primer
tgggtgtcgctgttgaagtc

SEQ ID NO: 45 - DNA, 22 bp, Artificial Sequence
  Primer
tggtcatccagcaggtgttcga

SEQ ID NO: 46 - DNA, 22 bp, Artificial Sequence
  Primer
acagacactggcaacattgcgg

SEQ ID NO: 47 - DNA, 20 bp, Artificial Sequence
  Primer
tccctggagaagagctacga

SEQ ID NO: 48 - DNA, 20 bp, Artificial Sequence
  Primer
agcactgtgttggcgtacag